European Patent Application EP 4 578 951 A1, published July 2, 2025. Title: MULTI-FRAGMENTED POLYA POLYNUCLEOTIDE STABLY EXISTING IN HOST CELL AND USE THEREOF. Applicant: SHENZHEN RHEGEN BIOTECHNOLOGY CO., LTD. Application EP 23856726.7, filed August 25, 2023. The sequence listing filed with the application follows.

SEQUENCE LISTING (81 sequences)

SEQ ID NO: 1 - DNA, 120 bp, synthetic construct
  source 1..120: mol_type = other DNA
aaaaaaaaaaaaaaaaaaaaaaaaaaaaaaaaaaaaaaaaaaaaaaaaaaaaaaaaaaaaaaaaaaaaaaaaaaaaaaaaaaaaaaaaaaaaaaaaaaaaaaaaaaaaaaaaaaaaaaaa

SEQ ID NO: 2 - DNA, 132 bp, synthetic construct
  source 1..132: mol_type = other DNA
aaaaaaaaaaaaaaaaaaaaaaaaaaaaaaaaaaaaaaaaatgcataaaaaaaaaaaaaaaaaaaaaaaaaaaaaaaaaaaaaaaagatatcaaaaaaaaaaaaaaaaaaaaaaaaaaaaaaaaaaaaaaaa

SEQ ID NO: 3 - DNA, 122 bp, synthetic construct
  source 1..122: mol_type = other DNA
aaaaaaaaaaaaaaaaaaaaaaaaaaaaaaaaaaaaaaaagaaaaaaaaaaaaaaaaaaaaaaaaaaaaaaaaaaaaaaaagaaaaaaaaaaaaaaaaaaaaaaaaaaaaaaaaaaaaaaaa

SEQ ID NO: 4 - DNA, 126 bp, synthetic construct
  source 1..126: mol_type = other DNA
aaaaaaaaaaaaaaaaaaaaaaaaaaaaaaaaaaaaaaaaaaaaaaaaaaaaaaaaaaaaatgcataaaaaaaaaaaaaaaaaaaaaaaaaaaaaaaaaaaaaaaaaaaaaaaaaaaaaaaaaaaa

SEQ ID NO: 5 - DNA, 132 bp, synthetic construct
  source 1..132: mol_type = other DNA
aaaaaaaaaaaaaaaaaaaaaaaaaaaaaaaaaaaaaaaaaaaaaaaaaaaaaaaaaaaacgccattagaggaaaaaaaaaaaaaaaaaaaaaaaaaaaaaaaaaaaaaaaaaaaaaaaaaaaaaaaaaaaa

SEQ ID NO: 6 - DNA, 144 bp, synthetic construct
  source 1..144: mol_type = other DNA
aaaaaaaaaaaaaaaaaaaaaaaaaaaaaaaaaaaaaaaaaaaaaaaaaaaaaaaaaaaacaacccctgattgtgtccgcatctaaaaaaaaaaaaaaaaaaaaaaaaaaaaaaaaaaaaaaaaaaaaaaaaaaaaaaaaaaaa

SEQ ID NO: 7 - DNA, 132 bp, synthetic construct
  source 1..132: mol_type = other DNA
aaaaaaaaaaaaaaaaaaaaaaaaaaaaaaaaaaaaaaaaaaaaaaaaaaaaaaaaaaaacctctaatggcgaaaaaaaaaaaaaaaaaaaaaaaaaaaaaaaaaaaaaaaaaaaaaaaaaaaaaaaaaaaa

SEQ ID NO: 8 - DNA, 132 bp, synthetic construct
  source 1..132: mol_type = other DNA
aaaaaaaaaaaaaaaaaaaaaaaaaaaaaaaaaaaaaaaaaaaaaaaaaaaaaaaaaaaaatgcatgatatcaaaaaaaaaaaaaaaaaaaaaaaaaaaaaaaaaaaaaaaaaaaaaaaaaaaaaaaaaaaa

SEQ ID NO: 9 - DNA, 132 bp, synthetic construct
  source 1..132: mol_type = other DNA
aaaaaaaaaaaaaaaaaaaaaaaaaaaaaaaaaaaaaaaaaaaaaaaaaaaaaaaaaaaatgcaacatcgataaaaaaaaaaaaaaaaaaaaaaaaaaaaaaaaaaaaaaaaaaaaaaaaaaaaaaaaaaaa

SEQ ID NO: 10 - DNA, 121 bp, synthetic construct
  source 1..121: mol_type = other DNA
aaaaaaaaaaaaaaaaaaaaaaaaaaaaaaaaaaaaaaaaaaaaaaaaaaaaaaaaaaaagaaaaaaaaaaaaaaaaaaaaaaaaaaaaaaaaaaaaaaaaaaaaaaaaaaaaaaaaaaaa

SEQ ID NO: 11 - DNA, 202 bp, synthetic construct
  source 1..202: mol_type = other DNA
aaaaaaaaaaaaaaaaaaaaaaaaaaaaaaaaaaaaaaaaaaaaaaaaaaaaaaaaaaaagaaaaaaaaaaaaaaaaaaaaaaaaaaaaaaaaaaaaaaaaaaaaaaaaaaaaaaaaaaaaaaaaaaaaaaaaaaaaaaaagaaaaaaaaaaaaaaaaaaaaaaaaaaaaaaaaaaaaaaaaaaaaaaaaaaaaaaaaaaaa

SEQ ID NO: 12 - DNA, 202 bp, synthetic construct
  source 1..202: mol_type = other DNA
aaaaaaaaaaaaaaaaaaaaaaaaaaaaaaaaaaaaaaaaaaaaaaaaaaaaaaaaaaaagaaaaaaaaaaaaaaaaaaaaaaaaaaaaaaaaaaaaaaaaaaaaaaaaaaaaaaaaaaaagaaaaaaaaaaaaaaaaaaaaaaaaaaaaaaaaaaaaaaaaaaaaaaaaaaaaaaaaaaaaaaaaaaaaaaaaaaaaaaaa

SEQ ID NO: 13 - DNA, 206 bp, synthetic construct
  source 1..206: mol_type = other DNA
aaaaaaaaaaaaaaaaaaaaaaaaaaaaaaaaaaaaaaaaaaaaaaaaaaaaaaaaaaaaaaaaaaaaaaaaaaaaaaaaaaaaaaaaaaaaaaaaaaaaggggggaaaaaaaaaaaaaaaaaaaaaaaaaaaaaaaaaaaaaaaaaaaaaaaaaaaaaaaaaaaaaaaaaaaaaaaaaaaaaaaaaaaaaaaaaaaaaaaaaaaa

SEQ ID NO: 14 - DNA, 206 bp, synthetic construct
  source 1..206: mol_type = other DNA
aaaaaaaaaaaaaaaaaaaaaaaaaaaaaaaaaaaaaaaaaaaaaaaaaaaaaaaaaaaaaaaaaaaaaaaaaaaaaaaaaaaaaaaaaaaaaaaaaaaaatgcataaaaaaaaaaaaaaaaaaaaaaaaaaaaaaaaaaaaaaaaaaaaaaaaaaaaaaaaaaaaaaaaaaaaaaaaaaaaaaaaaaaaaaaaaaaaaaaaaaaa

SEQ ID NO: 15 - DNA, 212 bp, synthetic construct
  source 1..212: mol_type = other DNA
aaaaaaaaaaaaaaaaaaaaaaaaaaaaaaaaaaaaaaaaaaaaaaaaaaaaaaaaaaaaaaaaaaaaaaaaaaaaaaaaaaaaaaaaaaaaaaaaaaaacgccattagaggaaaaaaaaaaaaaaaaaaaaaaaaaaaaaaaaaaaaaaaaaaaaaaaaaaaaaaaaaaaaaaaaaaaaaaaaaaaaaaaaaaaaaaaaaaaaaaaaaaaa

SEQ ID NO: 16 - DNA, 224 bp, synthetic construct
  source 1..224: mol_type = other DNA
aaaaaaaaaaaaaaaaaaaaaaaaaaaaaaaaaaaaaaaaaaaaaaaaaaaaaaaaaaaaaaaaaaaaaaaaaaaaaaaaaaaaaaaaaaaaaaaaaaaacaacccctgattgtgtccgcatctaaaaaaaaaaaaaaaaaaaaaaaaaaaaaaaaaaaaaaaaaaaaaaaaaaaaaaaaaaaaaaaaaaaaaaaaaaaaaaaaaaaaaaaaaaaaaaaaaaaa

SEQ ID NO: 17 - DNA, 201 bp, synthetic construct
  source 1..201: mol_type = other DNA
aaaaaaaaaaaaaaaaaaaaaaaaaaaaaaaaaaaaaaaaaaaaaaaaaaaaaaaaaaaaaaaaaaaaaaaaaaaaaaaaaaaaaaaaaaaaaaaaaaaagaaaaaaaaaaaaaaaaaaaaaaaaaaaaaaaaaaaaaaaaaaaaaaaaaaaaaaaaaaaaaaaaaaaaaaaaaaaaaaaaaaaaaaaaaaaaaaaaaaaa

SEQ ID NO: 18 - DNA, 212 bp, synthetic construct
  source 1..212: mol_type = other DNA
aaaaaaaaaaaaaaaaaaaaaaaaaaaaaaaaaaaaaaaaaaaaaaaaaaaaaaaaaaaaatgcataaaaaaaaaaaaaaaaaaaaaaaaaaaaaaaaaaaaaaaaaaaaaaaaaaaaaaaaaaaaaaaaaaaaaaaaaaaaaaaaatgcataaaaaaaaaaaaaaaaaaaaaaaaaaaaaaaaaaaaaaaaaaaaaaaaaaaaaaaaaaaa

SEQ ID NO: 19 - DNA, 212 bp, synthetic construct
  source 1..212: mol_type = other DNA
aaaaaaaaaaaaaaaaaaaaaaaaaaaaaaaaaaaaaaaaaaaaaaaaaaaaaaaaaaaaaaaaaaaaaaaaaaaaaaaaatgcataaaaaaaaaaaaaaaaaaaaaaaaaaaaaaaaaaaaaaaaaaaaaaaaaaaaaaaaaaaaatgcataaaaaaaaaaaaaaaaaaaaaaaaaaaaaaaaaaaaaaaaaaaaaaaaaaaaaaaaaaaa

SEQ ID NO: 20 - DNA, 212 bp, synthetic construct
  source 1..212: mol_type = other DNA
aaaaaaaaaaaaaaaaaaaaaaaaaaaaaaaaaaaaaaaaaaaaaaaaaaaaaaaaaaaaatgcataaaaaaaaaaaaaaaaaaaaaaaaaaaaaaaaaaaaaaaaaaaaaaaaaaaaaaaaaaaaatgcataaaaaaaaaaaaaaaaaaaaaaaaaaaaaaaaaaaaaaaaaaaaaaaaaaaaaaaaaaaaaaaaaaaaaaaaaaaaaaaa

SEQ ID NO: 21 - DNA, 172 bp, synthetic construct
  source 1..172: mol_type = other DNA
aaaaaaaaaaaaaaaaaaaaaaaaaaaaaaaaaaaaaaaaaaaaaaaaaaaaaaaaaaaaaaaaaaaaaaaaaaaaaaaacgccattagaggaaaaaaaaaaaaaaaaaaaaaaaaaaaaaaaaaaaaaaaaaaaaaaaaaaaaaaaaaaaaaaaaaaaaaaaaaaaaaaaa

SEQ ID NO: 22 - DNA, 170 bp, synthetic construct
  source 1..170: mol_type = other DNA
aaaaaaaaaaaaaaaaaaaaaaaaaaaaaaaaaaaaaaaaaaaaaaaaaaaaaaaaaaaaaaaaaaaaaaaaaaaaaaaagcatatgactaaaaaaaaaaaaaaaaaaaaaaaaaaaaaaaaaaaaaaaaaaaaaaaaaaaaaaaaaaaaaaaaaaaaaaaaaaaaaaaa

SEQ ID NO: 23 - DNA, 180 bp, synthetic construct
  source 1..180: mol_type = other DNA
aaaaaaaaaaaaaaaaaaaaaaaaaaaaaagcatatgactaaaaaaaaaaaaaaaaaaaaaaaaaaaaaaaaaaaaaaaaaaaaaaaaaaaaaaaaaaaaaaaaaaaaaaaaaaaaaaaaaaaaaaaaaaaaaaaaaaaagcatatgactaaaaaaaaaaaaaaaaaaaaaaaaaaaaaa

SEQ ID NO: 24 - DNA, 180 bp, synthetic construct
  source 1..180: mol_type = other DNA
aaaaaaaaaaaaaaaaaaaaaaaaaaaaaagcatatgactaaaaaaaaaaaaaaaaaaaaaaaaaaaaaagcatatgactaaaaaaaaaaaaaaaaaaaaaaaaaaaaaaaaaaaaaaaaaaaaaaaaaaaaaaaaaaaaaaaaaaaaaaaaaaaaaaaaaaaaaaaaaaaaaaaaaaaa

SEQ ID NO: 25 - DNA, 184 bp, synthetic construct
  source 1..184: mol_type = other DNA
aaaaaaaaaaaaaaaaaaaaaaaaaaaaaacgccattagaggaaaaaaaaaaaaaaaaaaaaaaaaaaaaaaaaaaaaaaaaaaaaaaaaaaaaaaaaaaaaaaaaaaaaaaaaaaaaaaaaaaaaaaaaaaaaaaaaaaaacgccattagaggaaaaaaaaaaaaaaaaaaaaaaaaaaaaaa

SEQ ID NO: 26 - DNA, 184 bp, synthetic construct
  source 1..184: mol_type = other DNA
aaaaaaaaaaaaaaaaaaaaaaaaaaaaaacgccattagaggaaaaaaaaaaaaaaaaaaaaaaaaaaaaaacgccattagaggaaaaaaaaaaaaaaaaaaaaaaaaaaaaaaaaaaaaaaaaaaaaaaaaaaaaaaaaaaaaaaaaaaaaaaaaaaaaaaaaaaaaaaaaaaaaaaaaaaaa

SEQ ID NO: 27 - DNA, 174 bp, synthetic construct
  source 1..174: mol_type = other DNA
aaaaaaaaaaaaaaaaaaaaaaaaaaaaaacgccattagaggaaaaaaaaaaaaaaaaaaaaaaaaaaaaaaaaaaaaaaaaaaaaaaaaaaaaaaaaaaaacgccattagaggaaaaaaaaaaaaaaaaaaaaaaaaaaaaaaaaaaaaaaaaaaaaaaaaaaaaaaaaaaaa

SEQ ID NO: 28 - DNA, 174 bp, synthetic construct
  source 1..174: mol_type = other DNA
aaaaaaaaaaaaaaaaaaaaaaaaaaaaaaaaaaaaaaaaaaaaaaaaaaaaaaaaaaaacgccattagaggaaaaaaaaaaaaaaaaaaaaaaaaaaaaaaaaaaaaaaaaaaaaaaaaaaaaaaaaaaaacgccattagaggaaaaaaaaaaaaaaaaaaaaaaaaaaaaaa

SEQ ID NO: 29 - DNA, 142 bp, synthetic construct
  source 1..142: mol_type = other DNA
aaaaaaaaaaaaaaaaaaaaaaaaaaaaaagcatatgactaaaaaaaaaaaaaaaaaaaaaaaaaaaaaaaaaaaaaaaaaaaaaaaaaaaaaaaaaaaacgccattagaggaaaaaaaaaaaaaaaaaaaaaaaaaaaaaa

SEQ ID NO: 30 - DNA, 172 bp, synthetic construct
  source 1..172: mol_type = other DNA
aaaaaaaaaaaaaaaaaaaaaaaaaaaaaaaaaaaaaaaaaaaaaaaaaaaaaaaaaaaaaaaaaaaaaaaaaaaaaaaacctctaatggcgaaaaaaaaaaaaaaaaaaaaaaaaaaaaaaaaaaaaaaaaaaaaaaaaaaaaaaaaaaaaaaaaaaaaaaaaaaaaaaaa

SEQ ID NO: 31 - DNA, 172 bp, synthetic construct
  source 1..172: mol_type = other DNA
aaaaaaaaaaaaaaaaaaaaaaaaaaaaaaaaaaaaaaaaaaaaaaaaaaaaaaaaaaaaaaaaaaaaaaaaaaaaaaaaatgcatgatatcaaaaaaaaaaaaaaaaaaaaaaaaaaaaaaaaaaaaaaaaaaaaaaaaaaaaaaaaaaaaaaaaaaaaaaaaaaaaaaaa

SEQ ID NO: 32 - DNA, 170 bp, synthetic construct
  source 1..170: mol_type = other DNA
aaaaaaaaaaaaaaaaaaaaaaaaaaaaaaaaaaaaaaaaaaaaaaaaaaaaaaaaaaaaaaaaaaaaaaaaaaaaaaaacagtaatgacaaaaaaaaaaaaaaaaaaaaaaaaaaaaaaaaaaaaaaaaaaaaaaaaaaaaaaaaaaaaaaaaaaaaaaaaaaaaaaaa

SEQ ID NO: 33 - DNA, 161 bp, synthetic construct
  source 1..161: mol_type = other DNA
aaaaaaaaaaaaaaaaaaaaaaaaaaaaaaaaaaaaaaaaaaaaaaaaaaaaaaaaaaaaaaaaaaaaaaaaaaaaaaaagaaaaaaaaaaaaaaaaaaaaaaaaaaaaaaaaaaaaaaaaaaaaaaaaaaaaaaaaaaaaaaaaaaaaaaaaaaaaaaaa

SEQ ID NO: 34 - DNA, 170 bp, synthetic construct
  source 1..170: mol_type = other DNA
aaaaaaaaaaaaaaaaaaaaaaaaaaaaaaaaaaaaaaaaaaaaaaaaaaaaaaaaaaaaaaaaaaaaaaaaaaaaaaaaagtcatatgcaaaaaaaaaaaaaaaaaaaaaaaaaaaaaaaaaaaaaaaaaaaaaaaaaaaaaaaaaaaaaaaaaaaaaaaaaaaaaaaa

SEQ ID NO: 35 - DNA, 170 bp, synthetic construct
  source 1..170: mol_type = other DNA
aaaaaaaaaaaaaaaaaaaaaaaaaaaaaaaaaaaaaaaaaaaaaaaaaaaaaaaaaaaaaaaaaaaaaaaaaaaaaaaagtcattactgaaaaaaaaaaaaaaaaaaaaaaaaaaaaaaaaaaaaaaaaaaaaaaaaaaaaaaaaaaaaaaaaaaaaaaaaaaaaaaaa

SEQ ID NO: 36 - DNA, 172 bp, synthetic construct
  source 1..172: mol_type = other DNA
aaaaaaaaaaaaaaaaaaaaaaaaaaaaaaaaaaaaaaaaaaaaaaaaaaaaaaaaaaaaaaaaaaaaaaaaaaaaaaaatgcaacatcgataaaaaaaaaaaaaaaaaaaaaaaaaaaaaaaaaaaaaaaaaaaaaaaaaaaaaaaaaaaaaaaaaaaaaaaaaaaaaaaa

SEQ ID NO: 37 - DNA, 172 bp, synthetic construct
  source 1..172: mol_type = other DNA
aaaaaaaaaaaaaaaaaaaaaaaaaaaaaagtcattactgaaaaaaaaaaaaaaaaaaaaaaaaaaaaaaaaaaaaaaaaaaaaaaaaaaaaaaaaaaaaatgcatgatatcaaaaaaaaaaaaaaaaaaaaaaaaaaaaaaaaaaaaaaaaaaaaaaaaaaaaaaaaaaaa

SEQ ID NO: 38 - DNA, 142 bp, synthetic construct
  source 1..142: mol_type = other DNA
aaaaaaaaaaaaaaaaaaaaaaaaaaaaaacgccattagaggaaaaaaaaaaaaaaaaaaaaaaaaaaaaaaaaaaaaaaaaaaaaaaaaaaaaaaaaaaaaaaaaaaaaaaaaaaaaaaaaaaaaaaaaaaaaaaaaaaaa

SEQ ID NO: 39 - DNA, 142 bp, synthetic construct
  source 1..142: mol_type = other DNA
aaaaaaaaaaaaaaaaaaaaaaaaaaaaaacctctaatggcgaaaaaaaaaaaaaaaaaaaaaaaaaaaaaaaaaaaaaaaaaaaaaaaaaaaaaaaaaaaaaaaaaaaaaaaaaaaaaaaaaaaaaaaaaaaaaaaaaaaa

SEQ ID NO: 40 - DNA, 140 bp, synthetic construct
  source 1..140: mol_type = other DNA
aaaaaaaaaaaaaaaaaaaaaaaaaaaaaagcatatgactaaaaaaaaaaaaaaaaaaaaaaaaaaaaaaaaaaaaaaaaaaaaaaaaaaaaaaaaaaaaaaaaaaaaaaaaaaaaaaaaaaaaaaaaaaaaaaaaaaaa

SEQ ID NO: 41 - DNA, 140 bp, synthetic construct
  source 1..140: mol_type = other DNA
aaaaaaaaaaaaaaaaaaaaaaaaaaaaaatgtcagatacaaaaaaaaaaaaaaaaaaaaaaaaaaaaaaaaaaaaaaaaaaaaaaaaaaaaaaaaaaaaaaaaaaaaaaaaaaaaaaaaaaaaaaaaaaaaaaaaaaaa

SEQ ID NO: 42 - DNA, 150 bp, synthetic construct
  source 1..150: mol_type = other DNA
aaaaaaaaaaaaaaaaaaaaaaaaaaaaaagcatatgactaaaaaaaaaaaaaaaaaaaaaaaaaaaaaagcatatgactaaaaaaaaaaaaaaaaaaaaaaaaaaaaaagcatatgactaaaaaaaaaaaaaaaaaaaaaaaaaaaaaa

SEQ ID NO: 43 - DNA, 150 bp, synthetic construct
  source 1..150: mol_type = other DNA
aaaaaaaaaaaaaaaaaaaaaaaaaaaaaatgtcagatacaaaaaaaaaaaaaaaaaaaaaaaaaaaaaatgtcagatacaaaaaaaaaaaaaaaaaaaaaaaaaaaaaatgtcagatacaaaaaaaaaaaaaaaaaaaaaaaaaaaaaa

SEQ ID NO: 44 - DNA, 110 bp, synthetic construct
  source 1..110: mol_type = other DNA
aaaaaaaaaaaaaaaaaaaaaaaaaaaaaagcatatgactaaaaaaaaaaaaaaaaaaaaaaaaaaaaaaaaaaaaaaaaaaaaaaaaaaaaaaaaaaaaaaaaaaaaaa

SEQ ID NO: 45 - DNA, 110 bp, synthetic construct
  source 1..110: mol_type = other DNA
aaaaaaaaaaaaaaaaaaaaaaaaaaaaaagctcatatgcaaaaaaaaaaaaaaaaaaaaaaaaaaaaaaaaaaaaaaaaaaaaaaaaaaaaaaaaaaaaaaaaaaaaaa

SEQ ID NO: 46 - DNA, 110 bp, synthetic construct
  source 1..110: mol_type = other DNA
aaaaaaaaaaaaaaaaaaaaaaaaaaaaaagcatatatgcaaaaaaaaaaaaaaaaaaaaaaaaaaaaaaaaaaaaaaaaaaaaaaaaaaaaaaaaaaaaaaaaaaaaaa

SEQ ID NO: 47 - DNA, 101 bp, synthetic construct
  source 1..101: mol_type = other DNA
aaaaaaaaaaaaaaaaaaaaaaaaaaaaaagaaaaaaaaaaaaaaaaaaaaaaaaaaaaaaaaaaaaaaaaaaaaaaaaaaaaaaaaaaaaaaaaaaaaaa

SEQ ID NO: 48 - DNA, 111 bp, synthetic construct
  source 1..111: mol_type = other DNA
aaaaaaaaaaaaaaaaaaaaaaaaaaaaaaaaaaaaaaaagaaaaaaaaaaaaaaaaaaaaaaaaaaaaaaaaaaaaaaaaaaaaaaaaaaaaaaaaaaaaaaaaaaaaaa

SEQ ID NO: 49 - DNA, 190 bp, synthetic construct
  source 1..190: mol_type = other DNA
aaaaaaaaaaaaaaaaaaaaaaaaaaaaaagcatatgactaaaaaaaaaaaaaaaaaaaaaaaaaaaaaaaaaaaaaaaaaaaaaaaaaaaaaaaaaaaaaaaaaaaaaagcatatgactaaaaaaaaaaaaaaaaaaaaaaaaaaaaaaaaaaaaaaaaaaaaaaaaaaaaaaaaaaaaaaaaaaaaaa

SEQ ID NO: 50 - DNA, 137 bp, synthetic construct
  source 1..137: mol_type = other DNA
aaaaaaaaaaaaaaacaaaaaaaaaaaaaaaaaaaaaaaaaaaaaaaaaaaaaaaaaaaaaaaaaaaaaaaaaaaaaaaaagaaaaaaaaaaaaaaaaaaaaaaaaaaaaaaaaaaaaaaaaaaaaaaaaaaaaaaa

SEQ ID NO: 51 - DNA, 130 bp, synthetic construct
  source 1..130: mol_type = other DNA
aaaaaaaaaaaaaaaaaaaaaaaaaaaaaaaaaaaaaaaagcatatgactaaaaaaaaaaaaaaaaaaaaaaaaaaaaaaaaaaaaaaaaaaaaaaaaaaaaaaaaaaaaaaaaaaaaaaaaaaaaaaaa

SEQ ID NO: 52 - DNA, 130 bp, synthetic construct
  source 1..130: mol_type = other DNA
aaaaaaaaaaaaaaaaaaaaaaaaaaaaaaaaaaaaaaaaaaaaaaaaaagcatatgactaaaaaaaaaaaaaaaaaaaaaaaaaaaaaaaaaaaaaaaaaaaaaaaaaaaaaaaaaaaaaaaaaaaaaa

SEQ ID NO: 53 - DNA, 10 bp, synthetic construct
  source 1..10: mol_type = other DNA
gcatatgact

SEQ ID NO: 54 - DNA, 10 bp, synthetic construct
  source 1..10: mol_type = other DNA
cagtaatgac

SEQ ID NO: 55 - DNA, 10 bp, synthetic construct
  source 1..10: mol_type = other DNA
agtcatatgc

SEQ ID NO: 56 - DNA, 10 bp, synthetic construct
  source 1..10: mol_type = other DNA
gtcattactg

SEQ ID NO: 57 - DNA, 10 bp, synthetic construct
  source 1..10: mol_type = other DNA
tgtcagatac

SEQ ID NO: 58 - DNA, 10 bp, synthetic construct
  source 1..10: mol_type = other DNA
gctcatatgc

SEQ ID NO: 59 - DNA, 10 bp, synthetic construct
  source 1..10: mol_type = other DNA
gcatatatgc

SEQ ID NO: 60 - DNA, 12 bp, synthetic construct
  source 1..12: mol_type = other DNA
cgccattagagg

SEQ ID NO: 61 - DNA, 12 bp, synthetic construct
  source 1..12: mol_type = other DNA
atgcatgatatc

SEQ ID NO: 62 - DNA, 12 bp, synthetic construct
  source 1..12: mol_type = other DNA
tgcaacatcgat

SEQ ID NO: 63 - DNA, 12 bp, synthetic construct
  source 1..12: mol_type = other DNA
cctctaatggcg

SEQ ID NO: 64 - DNA, 24 bp, synthetic construct
  source 1..24: mol_type = other DNA
caacccctgattgtgtccgcatct

SEQ ID NO: 65 - DNA, 19 bp, synthetic construct
  source 1..19: mol_type = other DNA
cgacggccagtgaattgac

SEQ ID NO: 66 - DNA, 20 bp, synthetic construct
  source 1..20: mol_type = other DNA
cagctatgaccatgctcgag

SEQ ID NO: 67 - DNA, 22 bp, synthetic construct
  source 1..22: mol_type = other DNA
tgagggtctagaactagtgtcg

SEQ ID NO: 68 - DNA, 25 bp, synthetic construct
  source 1..25: mol_type = other DNA
cttcctactcaggctttattcaaag

SEQ ID NO: 69 - DNA, 25 bp, synthetic construct
  source 1..25: mol_type = other DNA
ctttgaataaagcctgagtaggaag

SEQ ID NO: 70 - DNA, 22 bp, synthetic construct
  source 1..22: mol_type = other DNA
cgacactagttctagaccctca

SEQ ID NO: 71 - DNA, 25 bp, synthetic construct
  source 1..25: mol_type = other DNA
ctttgaataaagcctgagtaggaag

SEQ ID NO: 72 - DNA, 22 bp, synthetic construct
  source 1..22: mol_type = other DNA
cgacactagttctagaccctca

SEQ ID NO: 73 - DNA, 23 bp, synthetic construct
  source 1..23: mol_type = other DNA
gtacagaagctaatacgactcac

SEQ ID NO: 74 - DNA, 145 bp, synthetic construct
  source 1..145: mol_type = other DNA
ttttttttttttttttttttttttttttttttttttttttttttttttttttttttttttttttttttttttttttttttttttttttttttttttttttttttttttttttttttttttcttcctactcaggctttattcaaag

SEQ ID NO: 75 - DNA, 126 bp, synthetic construct
  source 1..126: mol_type = other DNA
ttttttttttttttttttttttttttttttttttttttttttttttttttttttttttttttttttttttcttttttttttttttttttttttttttttttcttcctactcaggctttattcaaag

SEQ ID NO: 76 - DNA, 150 bp, synthetic construct
  source 1..150: mol_type = other DNA
ttttttttttttttttttttttttttttttttttttttttttttttttttttttttttttttttttttttttttttttttagtcatatgcttttttttttttttttttttttttttttttttttttttttcttcctactcaggctttatt

SEQ ID NO: 77 - DNA, 100 bp, synthetic construct
  source 1..100: mol_type = other DNA
aaaaaaaaaaaaaaaaaaaaaaaaaaaaaagaaaaaaaaaaaaaaaaaaaaaaaaaaaaaaaaaaaaaaaaaaaaaaaaaaaaaaaaaaaaaaaaaaaaa

SEQ ID NO: 78 - DNA, 101 bp, synthetic construct; identical to SEQ ID NO: 47
  source 1..101: mol_type = other DNA

SEQ ID NO: 79 - DNA, 102 bp, synthetic construct
  source 1..102: mol_type = other DNA
aaaaaaaaaaaaaaaaaaaaaaaaaaaaaagaaaaaaaaaaaaaaaaaaaaaaaaaaaaaaaaaaaaaaaaaaaaaaaaaaaaaaaaaaaaaaaaaaaaaaa

SEQ ID NO: 80 - DNA, 100 bp, synthetic construct
  source 1..100: mol_type = other DNA
aaaaaaaaaaaaaaaaaaaaaaaaaaaaagaaaaaaaaaaaaaaaaaaaaaaaaaaaaaaaaaaaaaaaaaaaaaaaaaaaaaaaaaaaaaaaaaaaaaa

SEQ ID NO: 81 - DNA, 102 bp, synthetic construct
  source 1..102: mol_type = other DNA
aaaaaaaaaaaaaaaaaaaaaaaaaaaaaaagaaaaaaaaaaaaaaaaaaaaaaaaaaaaaaaaaaaaaaaaaaaaaaaaaaaaaaaaaaaaaaaaaaaaaa